European Patent Application EP 4 528 281 A2, published March 26, 2025. Title: Detection Method of Circulating BMP10 (Bone Morphogenetic Protein 10). Applicant: Universiteit Maastricht. The sequence listing filed with the application follows.

SEQUENCE LISTING (78 sequences)

SEQ ID NO: 1 - protein, 424 aa, Homo sapiens
MGSLVLTLCALFCLAAYLVSGSPIMNLEQSPLEEDMSLFGDVFSEQDGVDFNTLLQSMKDEFLKTLNLSDIPTQDSAKVDPPEYMLELYNKFATDRTSMPSANIIRSFKNEDLFSQPVSFNGLRKYPLLFNVSIPHHEEVIMAELRLYTLVQRDRMIYDGVDRKITIFEVLESKGDNEGERNMLVLVSGEIYGTNSEWETFDVTDAIRRWQKSGSSTHQLEVHIESKHDEAEDASSGRLEIDTSAQNKHNPLLIVFSDDQSSDKERKEELNEMISHEQLPELDNLGLDSFSSGPGEEALLQMRSNIIYDSTARIRRNAKGNYCKRTPLYIDFKEIGWDSWIIAPPGYEAYECRGVCNYPLAEHLTPTKHAIIQALVHLKNSQKASKACCVPTKLEPISILYLDKGVVTYKFKYEGMAVSECGCR

SEQ ID NO: 2 - protein, 11 aa, Homo sapiens
SLFGDVFSEQD

SEQ ID NO: 3 - protein, 15 aa, Homo sapiens
LESKGDNEGERNMLV

SEQ ID NO: 4 - protein, 9 aa, Homo sapiens
SKGDNEGER

SEQ ID NO: 5 - protein, 9 aa, Homo sapiens
SSGPGEEAL

SEQ ID NO: 6 - protein, 295 aa, Homo sapiens
SPIMNLEQSPLEEDMSLFGDVFSEQDGVDFNTLLQSMKDEFLKTLNLSDIPTQDSAKVDPPEYMLELYNKFATDRTSMPSANIIRSFKNEDLFSQPVSFNGLRKYPLLFNVSIPHHEEVIMAELRLYTLVQRDRMIYDGVDRKITIFEVLESKGDNEGERNMLVLVSGEIYGTNSEWETFDVTDAIRRWQKSGSSTHQLEVHIESKHDEAEDASSGRLEIDTSAQNKHNPLLIVFSDDQSSDKERKEELNEMISHEQLPELDNLGLDSFSSGPGEEALLQMRSNIIYDSTARIRR

SEQ ID NO: 7 - protein, 117 aa, synthetic construct
  REGION 1..117: note = VH-1
QSLEESGGRLVTPGTPLTLTCTVSGIDLSRNVMSWVRQAPGEGLEWIGSINTGGSTWYASWAEGRLTISKSSTTVDLKISSPTTEDTATYFCARGVYGHSNGYYSLWGQGTLVTVSS

SEQ ID NO: 8 - protein, 116 aa, synthetic construct
  REGION 1..116: note = VH-2
QSVEESGGRLVTPGTPLTLTCTASGFSLSSYAMSWVRQAPGKGLQFIGYISGGGSTYYASWVKGRFTISKTSTTVDLKLTSPTTEDTATYFCARGYPGYISGTWAVGQGTLVTVSS

SEQ ID NO: 9 - protein, 117 aa, synthetic construct
  REGION 1..117: note = VH-3
QSLEESGGRLVTPGTALTVTCTVSGIDLSRNLMSWVRQAPGEGLEWIGSINFRNITWYASWAKGRFTISKTSTTVDLRISSPTTEDTATYFCARGVYVNSNGYYSLWGQGTPVTVSS

SEQ ID NO: 10 - protein, 116 aa, synthetic construct
  REGION 1..116: note = VH-4
QSLEESGGRLVTPGTPLTLTCTVSGFSLSNYAMSWVRQAPGMGLEYIGYISASGNTYYASWVKGRFTISKTSTTVDLKMTSPTTEDTATYFCARGYSGWISGTWAVGQGTLVTVSS

SEQ ID NO: 11 - protein, 117 aa, synthetic construct
  REGION 1..117: note = VH-5
QSVEESGGRLVTPGTPLTLTCTASGIDLSRYAMTWVRQAPGKGLEWIGIIGASSGTWYASWAKGRFTIAKTSTTVDLRITSPTTEDTATYFCARDNGDSKDYAFDPWGPGTLVTVSS

SEQ ID NO: 12 - protein, 108 aa, synthetic construct
  REGION 1..108: note = VH-6
QSVEESGGRLVTPGTPLTLTCTASAFSLSRYVMSWVRQAPGKGLEFIGFINASGSTSYASWAKGRFTISKTSTTVDLKMTSLTTEDTATYFCATGNLWGPGTLVTVSS

SEQ ID NO: 13 - protein, 112 aa, synthetic construct
  REGION 1..112: note = VH-8
QSVEESGGRLVTPGTPLTLTCTASGFSLSKYDMSWVRQAPGKGLEWIGAIGGRGVTDYTTWAKGRFTISKTATTVDLKMTSPTTEDTATYFCVRALAGDTLWGPGTLVTVSS

SEQ ID NO: 14 - protein, 127 aa, synthetic construct
  REGION 1..127: note = VH-8
QSLEESGGDLVKPGASLTLTCTASGFSFSSSYWICWVRQAPGKGLEWIACIYAGSSDITYYASWAKGRFTVSKTSSPTVTLQMTSLTAADTATYFCARGRYYVDGYADYYPGDFNLWGPGTLVTVSS

SEQ ID NO: 15 - protein, 120 aa, synthetic construct
  REGION 1..120: note = VH-9
QSLEESGGGLVQPEGSLTLTCIASAFSFSSGYYMCWVRQAPGKGLEWIACIYAGSSGTTYYASWAKGRFTISKASSTTVTLLMTSLTAADTATYFCARGPGASGYRLGLWGPGTLVTVSS

SEQ ID NO: 16 - protein, 112 aa, synthetic construct
  REGION 1..112: note = VL-1
ALVMTQTPASVEAAVGGTVTINCQASQSISNLLAWYQQKPGQPPKVLIYAASPLASGVSPRFKGSGSGTHFTLTVSDLECADAATYYCQSYWGGSGERYLNTFGGGTEVVVK

SEQ ID NO: 17 - protein, 110 aa, synthetic construct
  REGION 1..110: note = VL-2
AVLTQTPSPVSAAVGGTVSISCQSSQSVVNNNRCSWFQQKPGQPPKQLIYSASTLASGVPSRFKGSGSGTQFTLTISDVQCDDAATYYCLGDYVSYGDSAFGGGTEVVVK

SEQ ID NO: 18 - protein, 112 aa, synthetic construct
  REGION 1..112: note = VL-3
DIVMTQTPASVEAAVGGTVTINCQASQSVSNLLAWYQQKPGQPPKLLIYGASKLESGVPSRFKGSGSGTQFTLTINDLECDDAATYYCQTYWGGDGTSYLNPFGGGTEVVVK

SEQ ID NO: 19 - protein, 110 aa, synthetic construct
  REGION 1..110: note = VL-4
AVLTQTPSPVSAAVGGTVNIGCQSSQSVVNNNRLSWFQQRPGQPPKQLIYRASTLASGVPSRFKGSGSGTQFTLTISDVQCDDAATYYCLGDYVSYSEAAFGGGTEVVVK

SEQ ID NO: 20 - protein, 109 aa, synthetic construct
  REGION 1..109: note = VL-5
IDMTQTPSPVSAAVGDTVTINCQASENIYSFLAWYQQKPGHSPNLLIYFASKLVSGVPSRFKGSGSGTQFTLTISDVQCDDAATYYCQQTYTYSNGDNPFGGGTEVVVK

SEQ ID NO: 21 - protein, 111 aa, synthetic construct
  REGION 1..111: note = VL-6
DIVMTQTPSSVSGPVGGTVTINCQASQNIYSNLAWYQQKPGQPPKLLIYYASTLVSGVPSRFKGSGSGTQFTLTISDLECANAATYYCQSKDGPTSSTYGAFGGGTEVVVR

SEQ ID NO: 22 - protein, 113 aa, synthetic construct
  REGION 1..113: note = VL-7
AQVLTQTASPVSAAVGSTVTINCQASQNIYKYNNLAWYQQKPGQPPKRLIYEASKLASGVPSRFSGSGSGTQFTLTISGVQCEDAATYYCQGTFECSSADCFGFGGGTEVVVK

SEQ ID NO: 23 - protein, 112 aa, synthetic construct
  REGION 1..112: note = VL-8
DIVMTQTPASVEAAVGGTVTIKCQASQSISSYLAWYQQKSGQPPKLLIYLASTLESGVPSRFKGSGSGTEFTLTISDLECADAATYYCQSYYYSSSSSYGSAFGGGTEVVVK

SEQ ID NO: 24 - protein, 109 aa, synthetic construct
  REGION 1..109: note = VL-9
DVVMTQTPASVSEPVGGTVTIKCQASEDIYRLLAWYQQKPGQPPKLLIYDASDLASGVPSRLSGSGSGTEYTLSISDLECADAATYYCQQGYYISGGDSFGGGTEVVVK

SEQ ID NO: 25 - protein, 5 aa, synthetic construct
  REGION 1..5: note = CDRH1-1
RNVMS

SEQ ID NO: 26 - protein, 5 aa, synthetic construct
  REGION 1..5: note = CDRH1-2
SYAMS

SEQ ID NO: 27 - protein, 5 aa, synthetic construct
  REGION 1..5: note = CDRH1-3
RNLMS

SEQ ID NO: 28 - protein, 5 aa, synthetic construct
  REGION 1..5: note = CDRH1-4
NYAMS

SEQ ID NO: 29 - protein, 5 aa, synthetic construct
  REGION 1..5: note = CDRH1-5
RYAMT

SEQ ID NO: 30 - protein, 5 aa, synthetic construct
  REGION 1..5: note = CDRH1-6
RYVMS

SEQ ID NO: 31 - protein, 5 aa, synthetic construct
  REGION 1..5: note = CDRH1-8
KYDMS

SEQ ID NO: 32 - protein, 7 aa, synthetic construct
  REGION 1..7: note = CDRH1-8
SSSYWIC

SEQ ID NO: 33 - protein, 7 aa, synthetic construct
  REGION 1..7: note = CDRH1-9
SSGYYMC

SEQ ID NO: 34 - protein, 11 aa, synthetic construct
  REGION 1..11: note = CDRL1-1
QASQSISNLLA

SEQ ID NO: 35 - protein, 13 aa, synthetic construct
  REGION 1..13: note = CDRL1-2
QSSQSVVNNNRCS

SEQ ID NO: 36 - protein, 11 aa, synthetic construct
  REGION 1..11: note = CDRL1-3
QASQSVSNLLA

SEQ ID NO: 37 - protein, 13 aa, synthetic construct
  REGION 1..13: note = CDRL1-4
QSSQSVVNNNRLS

SEQ ID NO: 38 - protein, 11 aa, synthetic construct
  REGION 1..11: note = CDRL1-5
QASENIYSFLA

SEQ ID NO: 39 - protein, 11 aa, synthetic construct
  REGION 1..11: note = CDRL1-6
QASQNIYSNLA

SEQ ID NO: 40 - protein, 13 aa, synthetic construct
  REGION 1..13: note = CDRL1-7
QASQNIYKYNNLA

SEQ ID NO: 41 - protein, 11 aa, synthetic construct
  REGION 1..11: note = CDRL1-8
QASQSISSYLA

SEQ ID NO: 42 - protein, 11 aa, synthetic construct
  REGION 1..11: note = CDRL1-9
QASEDIYRLLA

SEQ ID NO: 43 - protein, 16 aa, synthetic construct
  REGION 1..16: note = CDRH2-1
SINTGGSTWYASWAEG

SEQ ID NO: 44 - protein, 16 aa, synthetic construct
  REGION 1..16: note = CDRH2-2
YISGGGSTYYASWVKG

SEQ ID NO: 45 - protein, 16 aa, synthetic construct
  REGION 1..16: note = CDRH2-3
SINFRNITWYASWAKG

SEQ ID NO: 46 - protein, 16 aa, synthetic construct
  REGION 1..16: note = CDRH2-4
YISASGNTYYASWVKG

SEQ ID NO: 47 - protein, 16 aa, synthetic construct
  REGION 1..16: note = CDRH2-5
IIGASSGTWYASWAKG

SEQ ID NO: 48 - protein, 16 aa, synthetic construct
  REGION 1..16: note = CDRH2-6
FINASGSTSYASWAKG

SEQ ID NO: 49 - protein, 16 aa, synthetic construct
  REGION 1..16: note = CDRH2-7
AIGGRGVTDYTTWAKG

SEQ ID NO: 50 - protein, 18 aa, synthetic construct
  REGION 1..18: note = CDRH2-8
CIYAGSSDITYYASWAKG

SEQ ID NO: 51 - protein, 18 aa, synthetic construct
  REGION 1..18: note = CDRH2-9
CIYAGSSGTTYYASWAKG

SEQ ID NO: 52 - protein, 7 aa, synthetic construct
  REGION 1..7: note = CDRL2-1
AASPLAS

SEQ ID NO: 53 - protein, 7 aa, synthetic construct
  REGION 1..7: note = CDRL2-2
SASTLAS

SEQ ID NO: 54 - protein, 7 aa, synthetic construct
  REGION 1..7: note = CDRL2-3
GASKLES

SEQ ID NO: 55 - protein, 7 aa, synthetic construct
  REGION 1..7: note = CDRL2-5
RASTLAS

SEQ ID NO: 56 - protein, 7 aa, synthetic construct
  REGION 1..7: note = CDRL2-5
FASKLVS

SEQ ID NO: 57 - protein, 7 aa, synthetic construct
  REGION 1..7: note = CDRL2-6
YASTLVS

SEQ ID NO: 58 - protein, 7 aa, synthetic construct
  REGION 1..7: note = CDRL2-7
EASKLAS

SEQ ID NO: 59 - protein, 7 aa, synthetic construct
  REGION 1..7: note = CDRL2-8
LASTLES

SEQ ID NO: 60 - protein, 7 aa, synthetic construct
  REGION 1..7: note = CDRL2-9
DASDLAS

SEQ ID NO: 61 - protein, 12 aa, synthetic construct
  REGION 1..12: note = CDRH3-1
GVYGHSNGYYSL

SEQ ID NO: 62 - protein, 11 aa, synthetic construct
  REGION 1..11: note = CDRH3-2
GYPGYISGTWA

SEQ ID NO: 63 - protein, 12 aa, synthetic construct
  REGION 1..12: note = CDRH3-4
GVYVNSNGYYSL

SEQ ID NO: 64 - protein, 11 aa, synthetic construct
  REGION 1..11: note = CDRH3-4
GYSGWISGTWA

SEQ ID NO: 65 - protein, 12 aa, synthetic construct
  REGION 1..12: note = CDRH3-5
DNGDSKDYAFDP

SEQ ID NO: 66 - skipped

SEQ ID NO: 67 - protein, 7 aa, synthetic construct
  REGION 1..7: note = CDRH3-7
ALAGDTL

SEQ ID NO: 68 - protein, 18 aa, synthetic construct
  REGION 1..18: note = CDRH3-8
GRYYVDGYADYYPGDFNL

SEQ ID NO: 69 - protein, 11 aa, synthetic construct
  REGION 1..11: note = CDRH3-9
GPGASGYRLGL

SEQ ID NO: 70 - protein, 14 aa, synthetic construct
  REGION 1..14: note = CDRL3-1
QSYWGGSGERYLNT

SEQ ID NO: 71 - protein, 11 aa, synthetic construct
  REGION 1..11: note = CDRL3-2
LGDYVSYGDSA

SEQ ID NO: 72 - protein, 14 aa, synthetic construct
  REGION 1..14: note = CDRL3-3
QTYWGGDGTSYLNP

SEQ ID NO: 73 - protein, 11 aa, synthetic construct
  REGION 1..11: note = CDRL3-5
LGDYVSYSEAA

SEQ ID NO: 74 - protein, 12 aa, synthetic construct
  REGION 1..12: note = CDRL3-5
QQTYTYSNGDNP

SEQ ID NO: 75 - protein, 13 aa, synthetic construct
  REGION 1..13: note = CDRL3-8
QSKDGPTSSTYGA

SEQ ID NO: 76 - protein, 13 aa, synthetic construct
  REGION 1..13: note = CDRL3-7
QGTFECSSADCFG

SEQ ID NO: 77 - protein, 14 aa, synthetic construct
  REGION 1..14: note = CDRL3-8
QSYYYSSSSSYGSA

SEQ ID NO: 78 - protein, 11 aa, synthetic construct
  REGION 1..11: note = CDRL3-9
QQGYYISGGDS